European Patent Application EP 4 663 240 A1, published December 17, 2025. Title: IFN-γ PATHWAY INHIBITORS FOR USE IN THE TREATMENT OF FSHD. Applicant: Ospedale San Raffaele S.r.l. Application EP, filed June 12, 2024. The sequence listing filed with the application follows.

SEQUENCE LISTING (48 sequences)

SEQ ID NO: 1 - DNA, 24 bp, synthetic construct
  source 1..24: mol_type = other DNA
cttccgtgaaattctggctgaatg

SEQ ID NO: 2 - DNA, 33 bp, synthetic construct
  source 1..33: mol_type = other DNA
tttttttttttttttttctataggatccacagg

SEQ ID NO: 3 - DNA, 22 bp, synthetic construct
  source 1..22: mol_type = other DNA
ttggtgattccactggatttct

SEQ ID NO: 4 - DNA, 22 bp, synthetic construct
  source 1..22: mol_type = other DNA
tcggatggaatcaatgaaggga

SEQ ID NO: 5 - DNA, 22 bp, synthetic construct
  source 1..22: mol_type = other DNA
attggcaacaccgtattctgct

SEQ ID NO: 6 - DNA, 23 bp, synthetic construct
  source 1..23: mol_type = other DNA
cagtcaaaatatggacggatggt

SEQ ID NO: 7 - DNA, 20 bp, synthetic construct
  source 1..20: mol_type = other DNA
atatcctgcctggatggggt

SEQ ID NO: 8 - DNA, 22 bp, synthetic construct
  source 1..22: mol_type = other DNA
gagcttcttagtcctcctgtgt

SEQ ID NO: 9 - DNA, 21 bp, synthetic construct
  source 1..21: mol_type = other DNA
tggttgggccacctagaagta

SEQ ID NO: 10 - DNA, 19 bp, synthetic construct
  source 1..19: mol_type = other DNA
tctccattcctggcctgtg

SEQ ID NO: 11 - DNA, 22 bp, synthetic construct
  source 1..22: mol_type = other DNA
gagcaacttctttcaaccacag

SEQ ID NO: 12 - DNA, 21 bp, synthetic construct
  source 1..21: mol_type = other DNA
cacttccttctgccaaacttg

SEQ ID NO: 13 - DNA, 23 bp, synthetic construct
  source 1..23: mol_type = other DNA
ccagcattactagtcagaaggaa

SEQ ID NO: 14 - DNA, 21 bp, synthetic construct
  source 1..21: mol_type = other DNA
cacagtgcaatcttgtcatcc

SEQ ID NO: 15 - DNA, 20 bp, synthetic construct
  source 1..20: mol_type = other DNA
gggagagattgaccagcagt

SEQ ID NO: 16 - DNA, 20 bp, synthetic construct
  source 1..20: mol_type = other DNA
tgattcttcccacaggcacc

SEQ ID NO: 17 - DNA, 23 bp, synthetic construct
  source 1..23: mol_type = other DNA
cattcagatgtagcggataatgg

SEQ ID NO: 18 - DNA, 21 bp, synthetic construct
  source 1..21: mol_type = other DNA
cactcttttggatgctctggt

SEQ ID NO: 19 - DNA, 20 bp, synthetic construct
  source 1..20: mol_type = other DNA
cttggatcagctgcagaact

SEQ ID NO: 20 - DNA, 20 bp, synthetic construct
  source 1..20: mol_type = other DNA
gtgcggtcccataacacttg

SEQ ID NO: 21 - DNA, 18 bp, synthetic construct
  source 1..18: mol_type = other DNA
ccagaacagatttgagag

SEQ ID NO: 22 - DNA, 18 bp, synthetic construct
  source 1..18: mol_type = other DNA
ctacatttgccgaagagc

SEQ ID NO: 23 - DNA, 19 bp, synthetic construct
  source 1..19: mol_type = other DNA
agtttgaggtgagacggca

SEQ ID NO: 24 - DNA, 20 bp, synthetic construct
  source 1..20: mol_type = other DNA
tcccaatctgtctgcagtgg

SEQ ID NO: 25 - DNA, 20 bp, synthetic construct
  source 1..20: mol_type = other DNA
atgacctcctctcacagctg

SEQ ID NO: 26 - DNA, 23 bp, synthetic construct
  source 1..23: mol_type = other DNA
cctttcttccttcagacagttgt

SEQ ID NO: 27 - DNA, 21 bp, synthetic construct
  source 1..21: mol_type = other DNA
gcaatatagccgattcctgca

SEQ ID NO: 28 - DNA, 18 bp, synthetic construct
  source 1..18: mol_type = other DNA
tctggaggaggcgagact

SEQ ID NO: 29 - DNA, 19 bp, synthetic construct
  source 1..19: mol_type = other DNA
agctgcaggtccaagagcg

SEQ ID NO: 30 - DNA, 21 bp, synthetic construct
  source 1..21: mol_type = other DNA
ggtggtcagggctgagtcatt

SEQ ID NO: 31 - DNA, 21 bp, synthetic construct
  source 1..21: mol_type = other DNA
ggtgtccgtgactaactccat

SEQ ID NO: 32 - DNA, 21 bp, synthetic construct
  source 1..21: mol_type = other DNA
tggaaagggtaagaccgtcct

SEQ ID NO: 33 - DNA, 19 bp, synthetic construct
  source 1..19: mol_type = other DNA
caggagctgtacggcttcc

SEQ ID NO: 34 - DNA, 23 bp, synthetic construct
  source 1..23: mol_type = other DNA
cctaccttgagtaccttgagcac

SEQ ID NO: 35 - DNA, 21 bp, synthetic construct
  source 1..21: mol_type = other DNA
ggagaggagacttcacagagg

SEQ ID NO: 36 - DNA, 20 bp, synthetic construct
  source 1..20: mol_type = other DNA
ccagtttggtagcatccatc

SEQ ID NO: 37 - DNA, 20 bp, synthetic construct
  source 1..20: mol_type = other DNA
accacaatggtgctgttgaa

SEQ ID NO: 38 - DNA, 20 bp, synthetic construct
  source 1..20: mol_type = other DNA
aatctctggggcaaaggtct

SEQ ID NO: 39 - DNA, 20 bp, synthetic construct
  source 1..20: mol_type = other DNA
ccccacaaggctagtctcat

SEQ ID NO: 40 - DNA, 20 bp, synthetic construct
  source 1..20: mol_type = other DNA
gtcccgtgtcgttttacctg

SEQ ID NO: 41 - DNA, 20 bp, synthetic construct
  source 1..20: mol_type = other DNA
agacattcctgaggctgctt

SEQ ID NO: 42 - DNA, 20 bp, synthetic construct
  source 1..20: mol_type = other DNA
aggagacagtggattcgacc

SEQ ID NO: 43 - DNA, 24 bp, synthetic construct
  source 1..24: mol_type = other DNA
cttgcccttaaaggtctaaaagca

SEQ ID NO: 44 - DNA, 29 bp, synthetic construct
  source 1..29: mol_type = other DNA
gcggtataaggtacaattaaaagatatgg

SEQ ID NO: 45 - DNA, 18 bp, synthetic construct
  source 1..18: mol_type = other DNA
ggcctggacgacaaaacc

SEQ ID NO: 46 - DNA, 18 bp, synthetic construct
  source 1..18: mol_type = other DNA
caggatgggctccatgac

SEQ ID NO: 47 - DNA, 20 bp, synthetic construct
  source 1..20: mol_type = other DNA
cctcagggtattgctggaca

SEQ ID NO: 48 - DNA, 20 bp, synthetic construct
  source 1..20: mol_type = other DNA
gaaggaccttgtttgccagg